European Patent Application EP 4 407 031 A2, published July 31, 2024. Title: APTÂMERO DE ÁCIDO NUCLEICO, COMPOSIÇÃO, USO DE UM APTÂMERO, KIT DIAGNÓSTICO, MÉTODO IN VITRO PARA DETECTAR OU DIAGNOSTICAR UM TUMOR, E, MÉTODO PARA TRATAMENTO DE CÂNCER. Applicant: Fundação Oswaldo Cruz. The sequence listing filed with the application follows.

SEQUENCE LISTING (60 sequences)

SEQ ID NO: 1 - DNA, 30 bp, synthetic construct
  source 1..30: mol_type = other DNA
catacactctttatactctcatattaacca

SEQ ID NO: 2 - DNA, 30 bp, synthetic construct
  source 1..30: mol_type = other DNA
tcccattctctataatagtcccccactata

SEQ ID NO: 3 - DNA, 31 bp, synthetic construct
  source 1..31: mol_type = other DNA
acgctaatatctgattaattacttttttttg

SEQ ID NO: 4 - DNA, 30 bp, synthetic construct
  source 1..30: mol_type = other DNA
ggtgtagttatttgatattctttattgctg

SEQ ID NO: 5 - DNA, 30 bp, synthetic construct
  source 1..30: mol_type = other DNA
tgggattagtttatgttgtttgttgttatt

SEQ ID NO: 6 - DNA, 30 bp, synthetic construct
  source 1..30: mol_type = other DNA
cacggatataattatacccttttagtttga

SEQ ID NO: 7 - DNA, 30 bp, synthetic construct
  source 1..30: mol_type = other DNA
caatacactctttataaacgtttcctttca

SEQ ID NO: 8 - DNA, 30 bp, synthetic construct
  source 1..30: mol_type = other DNA
gtattgttttgttgtttcttgtataattcg

SEQ ID NO: 9 - DNA, 30 bp, synthetic construct
  source 1..30: mol_type = other DNA
tggtagtataggttgttgttggtatttata

SEQ ID NO: 10 - DNA, 30 bp, synthetic construct
  source 1..30: mol_type = other DNA
tagcgttttataaatctctcctttattgtg

SEQ ID NO: 11 - DNA, 76 bp, synthetic construct
  source 1..76: mol_type = other DNA
tagggaagagaaggacatatgatcatacactctttatactctcatattaaccattgactagtacatgaccacttga

SEQ ID NO: 12 - DNA, 76 bp, synthetic construct
  source 1..76: mol_type = other DNA
tagggaagagaaggacatatgattcccattctctataatagtcccccactatattgactagtacatgaccacttga

SEQ ID NO: 13 - DNA, 77 bp, synthetic construct
  source 1..77: mol_type = other DNA
tagggaagagaaggacatatgatacgctaatatctgattaattacttttttttgttgactagtacatgaccacttga

SEQ ID NO: 14 - DNA, 76 bp, synthetic construct
  source 1..76: mol_type = other DNA
tagggaagagaaggacatatgatggtgtagttatttgatattctttattgctgttgactagtacatgaccacttga

SEQ ID NO: 15 - DNA, 76 bp, synthetic construct
  source 1..76: mol_type = other DNA
tagggaagagaaggacatatgattgggattagtttatgttgtttgttgttattttgactagtacatgaccacttga

SEQ ID NO: 16 - DNA, 76 bp, synthetic construct
  source 1..76: mol_type = other DNA
tagggaagagaaggacatatgatcacggatataattatacccttttagtttgattgactagtacatgaccacttga

SEQ ID NO: 17 - DNA, 76 bp, synthetic construct
  source 1..76: mol_type = other DNA
tagggaagagaaggacatatgatcaatacactctttataaacgtttcctttcattgactagtacatgaccacttga

SEQ ID NO: 18 - DNA, 76 bp, synthetic construct
  source 1..76: mol_type = other DNA
tagggaagagaaggacatatgatgtattgttttgttgtttcttgtataattcgttgactagtacatgaccacttga

SEQ ID NO: 19 - DNA, 76 bp, synthetic construct
  source 1..76: mol_type = other DNA
tagggaagagaaggacatatgattggtagtataggttgttgttggtatttatattgactagtacatgaccacttga

SEQ ID NO: 20 - DNA, 76 bp, synthetic construct
  source 1..76: mol_type = other DNA
tagggaagagaaggacatatgattagcgttttataaatctctcctttattgtgttgactagtacatgaccacttga

SEQ ID NO: 21 - DNA, 30 bp, synthetic construct
  source 1..30: mol_type = other DNA
acgagatctcgaggtaagtcatacttcgca

SEQ ID NO: 22 - DNA, 30 bp, synthetic construct
  source 1..30: mol_type = other DNA
gtcacgaatatgatgaggctgacatgtcgg

SEQ ID NO: 23 - DNA, 30 bp, synthetic construct
  source 1..30: mol_type = other DNA
cgaattgtcgaacgaggctcctccgaggat

SEQ ID NO: 24 - DNA, 30 bp, synthetic construct
  source 1..30: mol_type = other DNA
gctacgagttttgaggttttgcatggttcg

SEQ ID NO: 25 - DNA, 32 bp, synthetic construct
  source 1..32: mol_type = other DNA
gctacgagtttttgaggtttttgcatggttcg

SEQ ID NO: 26 - DNA, 30 bp, synthetic construct
  source 1..30: mol_type = other DNA
acgagtgtaccgaggttaagtcacttggtc

SEQ ID NO: 27 - DNA, 30 bp, synthetic construct
  source 1..30: mol_type = other DNA
acgcagtgcgaatgaggttaatcatttctc

SEQ ID NO: 28 - DNA, 30 bp, synthetic construct
  source 1..30: mol_type = other DNA
ggagtaagagcaccccggaccgcgcgaccg

SEQ ID NO: 29 - DNA, 30 bp, synthetic construct
  source 1..30: mol_type = other DNA
cgtagaacctgggatgcatttcagcgagta

SEQ ID NO: 30 - DNA, 31 bp, synthetic construct
  source 1..31: mol_type = other DNA
gcaacccgtccccccactaatttacgcatca

SEQ ID NO: 31 - DNA, 76 bp, synthetic construct
  source 1..76: mol_type = other DNA
tagggaagagaaggacatatgatacgagatctcgaggtaagtcatacttcgcattgactagtacatgaccacttga

SEQ ID NO: 32 - DNA, 76 bp, synthetic construct
  source 1..76: mol_type = other DNA
tagggaagagaaggacatatgatgtcacgaatatgatgaggctgacatgtcggttgactagtacatgaccacttga

SEQ ID NO: 33 - DNA, 76 bp, synthetic construct
  source 1..76: mol_type = other DNA
tagggaagagaaggacatatgatcgaattgtcgaacgaggctcctccgaggatttgactagtacatgaccacttga

SEQ ID NO: 34 - DNA, 76 bp, synthetic construct
  source 1..76: mol_type = other DNA
tagggaagagaaggacatatgatgctacgagttttgaggttttgcatggttcgttgactagtacatgaccacttga

SEQ ID NO: 35 - DNA, 78 bp, synthetic construct
  source 1..78: mol_type = other DNA
tagggaagagaaggacatatgatgctacgagtttttgaggtttttgcatggttcgttgactagtacatgaccacttga

SEQ ID NO: 36 - DNA, 76 bp, synthetic construct
  source 1..76: mol_type = other DNA
tagggaagagaaggacatatgatacgagtgtaccgaggttaagtcacttggtcttgactagtacatgaccacttga

SEQ ID NO: 37 - DNA, 76 bp, synthetic construct
  source 1..76: mol_type = other DNA
tagggaagagaaggacatatgatacgcagtgcgaatgaggttaatcatttctcttgactagtacatgaccacttga

SEQ ID NO: 38 - DNA, 76 bp, synthetic construct
  source 1..76: mol_type = other DNA
tagggaagagaaggacatatgatggagtaagagcaccccggaccgcgcgaccgttgactagtacatgaccacttga

SEQ ID NO: 39 - DNA, 76 bp, synthetic construct
  source 1..76: mol_type = other DNA
tagggaagagaaggacatatgatcgtagaacctgggatgcatttcagcgagtattgactagtacatgaccacttga

SEQ ID NO: 40 - DNA, 77 bp, synthetic construct
  source 1..77: mol_type = other DNA
tagggaagagaaggacatatgatgcaacccgtccccccactaatttacgcatcattgactagtacatgaccacttga

SEQ ID NO: 41 - DNA, 30 bp, synthetic construct
  source 1..30: mol_type = other DNA
gcacgtcccccactccaactaatcgcatca

SEQ ID NO: 42 - DNA, 30 bp, synthetic construct
  source 1..30: mol_type = other DNA
agacaacgcgtcccccactaacccctgtcg

SEQ ID NO: 43 - DNA, 30 bp, synthetic construct
  source 1..30: mol_type = other DNA
cgggttgtagtggtggccccataccgtatt

SEQ ID NO: 44 - DNA, 31 bp, synthetic construct
  source 1..31: mol_type = other DNA
ccccacccccccctctttgcagttgctctgg

SEQ ID NO: 45 - DNA, 30 bp, synthetic construct
  source 1..30: mol_type = other DNA
caccgtcccccactgcatcacgatcgtatg

SEQ ID NO: 46 - DNA, 30 bp, synthetic construct
  source 1..30: mol_type = other DNA
gggctaggcaaaccccgtcccccactctat

SEQ ID NO: 47 - DNA, 30 bp, synthetic construct
  source 1..30: mol_type = other DNA
cgcggctccgaaagctcgtttacccccgac

SEQ ID NO: 48 - DNA, 31 bp, synthetic construct
  source 1..31: mol_type = other DNA
cagccccagtccccccactcattgttgatca

SEQ ID NO: 49 - DNA, 30 bp, synthetic construct
  source 1..30: mol_type = other DNA
cgggtgttttatgcggaggggtgttacgga

SEQ ID NO: 50 - DNA, 30 bp, synthetic construct
  source 1..30: mol_type = other DNA
gtcgcgggagagtttttgcaattgatgctg

SEQ ID NO: 51 - DNA, 76 bp, synthetic construct
  source 1..76: mol_type = other DNA
tagggaagagaaggacatatgatgcacgtcccccactccaactaatcgcatcattgactagtacatgaccacttga

SEQ ID NO: 52 - DNA, 76 bp, synthetic construct
  source 1..76: mol_type = other DNA
tagggaagagaaggacatatgatagacaacgcgtcccccactaacccctgtcgttgactagtacatgaccacttga

SEQ ID NO: 53 - DNA, 76 bp, synthetic construct
  source 1..76: mol_type = other DNA
tagggaagagaaggacatatgatcgggttgtagtggtggccccataccgtattttgactagtacatgaccacttga

SEQ ID NO: 54 - DNA, 77 bp, synthetic construct
  source 1..77: mol_type = other DNA
tagggaagagaaggacatatgatccccacccccccctctttgcagttgctctggttgactagtacatgaccacttga

SEQ ID NO: 55 - DNA, 76 bp, synthetic construct
  source 1..76: mol_type = other DNA
tagggaagagaaggacatatgatcaccgtcccccactgcatcacgatcgtatgttgactagtacatgaccacttga

SEQ ID NO: 56 - DNA, 76 bp, synthetic construct
  source 1..76: mol_type = other DNA
tagggaagagaaggacatatgatgggctaggcaaaccccgtcccccactctatttgactagtacatgaccacttga

SEQ ID NO: 57 - DNA, 76 bp, synthetic construct
  source 1..76: mol_type = other DNA
tagggaagagaaggacatatgatcgcggctccgaaagctcgtttacccccgacttgactagtacatgaccacttga

SEQ ID NO: 58 - DNA, 77 bp, synthetic construct
  source 1..77: mol_type = other DNA
tagggaagagaaggacatatgatcagccccagtccccccactcattgttgatcattgactagtacatgaccacttga

SEQ ID NO: 59 - DNA, 76 bp, synthetic construct
  source 1..76: mol_type = other DNA
tagggaagagaaggacatatgatcgggtgttttatgcggaggggtgttacggattgactagtacatgaccacttga

SEQ ID NO: 60 - DNA, 76 bp, synthetic construct
  source 1..76: mol_type = other DNA
tagggaagagaaggacatatgatgtcgcgggagagtttttgcaattgatgctgttgactagtacatgaccacttga